European Patent Application EP 4 477 672 A1, published December 18, 2024. Title: 一种新型双特异性嵌合抗原受体的构建及其应用. Applicant: 北京大学深圳研究生院. The sequence listing filed with the application follows.

SEQUENCE LISTING (13 sequences)

SEQ ID NO: 1 - protein, 616 aa, synthetic construct
MALPVTALLLPLALLLHAARPEVQLVESGGGLVQGGGSLRVSCVASGLSFSLYGMGWFRQAPGKEREFVAAINWRGDSTSYADSVKGRFTISRENAKNTAYLQMNSLKPEDTAVYYCAARKYSAANVFKPNDYDYWGQGTQVTVSSGGGGSDIQMTQTTSSLSASLGDRVTISCRASQDISKYLNWYQQKPDGTVKLLIYHTSRLHSGVPSRFSGSGSGTDYSLTISNLEQEDIATYFCQQGNTLPYTFGGGTKLEITGGGGSGGGGSGGGGSEVKLQESGPGLVAPSQSLSVTCTVSGVSLPDYGVSWIRQPPRKGLEWLGVIWGSETTYYNSALKSRLTIIKDNSKSQVFLKMNSLQTDDTAIYYCAKHYYYGGSYAMDYWGQGTSVTVSSTTTPAPRPPTPAPTIASQPLSLRPEACRPAAGGAVHTRGLDFACDIYIWAPLAGTCGVLLLSLVITLYCKRGRKKLLYIFKQPFMRPVQTTQEEDGCSCRFPEEEEGGCELRVKFSRSADAPAYKQGQNQLYNELNLGRREEYDVLDKRRGRDPEMGGKPRRKNPQEGLYNELQKDKMAEAYSEIGMKGERRRGKGHDGLYQGLSTATKDTYDALHMQALPPR

SEQ ID NO: 2 - protein, 640 aa, synthetic construct
MALPVTALLLPLALLLHAARPEVQLVESGGGLVQGGGSLRVSCVASGLSFSLYGMGWFRQAPGKEREFVAAINWRGDSTSYADSVKGRFTISRENAKNTAYLQMNSLKPEDTAVYYCAARKYSAANVFKPNDYDYWGQGTQVTVSSEPKIPQPQPKPQPQPQPQPQPKPQPKPEPDIQMTQTTSSLSASLGDRVTISCRASQDISKYLNWYQQKPDGTVKLLIYHTSRLHSGVPSRFSGSGSGTDYSLTISNLEQEDIATYFCQQGNTLPYTFGGGTKLEITGGGGSGGGGSGGGGSEVKLQESGPGLVAPSQSLSVTCTVSGVSLPDYGVSWIRQPPRKGLEWLGVIWGSETTYYNSALKSRLTIIKDNSKSQVFLKMNSLQTDDTAIYYCAKHYYYGGSYAMDYWGQGTSVTVSSTTTPAPRPPTPAPTIASQPLSLRPEACRPAAGGAVHTRGLDFACDIYIWAPLAGTCGVLLLSLVITLYCKRGRKKLLYIFKQPFMRPVQTTQEEDGCSCRFPEEEEGGCELRVKFSRSADAPAYKQGQNQLYNELNLGRREEYDVLDKRRGRDPEMGGKPRRKNPQEGLYNELQKDKMAEAYSEIGMKGERRRGKGHDGLYQGLSTATKDTYDALHMQALPPR

SEQ ID NO: 3 - protein, 612 aa, synthetic construct
MALPVTALLLPLALLLHAARPDIQMTQTTSSLSASLGDRVTISCRASQDISKYLNWYQQKPDGTVKLLIYHTSRLHSGVPSRFSGSGSGTDYSLTISNLEQEDIATYFCQQGNTLPYTFGGGTKLEITEETKKYQSEVQLVESGGGLVQGGGSLRVSCVASGLSFSLYGMGWFRQAPGKEREFVAAINWRGDSTSYADSVKGRFTISRENAKNTAYLQMNSLKPEDTAVYYCAARKYSAANVFKPNDYDYWGQGTQVTVSSSYTYNYEKEVKLQESGPGLVAPSQSLSVTCTVSGVSLPDYGVSWIRQPPRKGLEWLGVIWGSETTYYNSALKSRLTIIKDNSKSQVFLKMNSLQTDDTAIYYCAKHYYYGGSYAMDYWGQGTSVTVSSTTTPAPRPPTPAPTIASQPLSLRPEACRPAAGGAVHTRGLDFACDIYIWAPLAGTCGVLLLSLVITLYCKRGRKKLLYIFKQPFMRPVQTTQEEDGCSCRFPEEEEGGCELRVKFSRSADAPAYKQGQNQLYNELNLGRREEYDVLDKRRGRDPEMGGKPRRKNPQEGLYNELQKDKMAEAYSEIGMKGERRRGKGHDGLYQGLSTATKDTYDALHMQALPPR

SEQ ID NO: 4 - protein, 611 aa, synthetic construct
MALPVTALLLPLALLLHAARPDIQMTQTTSSLSASLGDRVTISCRASQDISKYLNWYQQKPDGTVKLLIYHTSRLHSGVPSRFSGSGSGTDYSLTISNLEQEDIATYFCQQGNTLPYTFGGGTKLEITEETKKYQSEVQLVESGGGLVQAGGSLRLSCAASGLTFNTYYMGWFRQPPGKEREFVARISASGASTDYADSVKGRFTISRDNAKNTMYLQMSSLKPEDTAVYYCEADRYGLRYSPVDVYPYWGQGTQVTVSSSYTYNYEKEVKLQESGPGLVAPSQSLSVTCTVSGVSLPDYGVSWIRQPPRKGLEWLGVIWGSETTYYNSALKSRLTIIKDNSKSQVFLKMNSLQTDDTAIYYCAKHYYYGGSYAMDYWGQGTSVTVSSTTTPAPRPPTPAPTIASQPLSLRPEACRPAAGGAVHTRGLDFACDIYIWAPLAGTCGVLLLSLVITLYCKRGRKKLLYIFKQPFMRPVQTTQEEDGCSCRFPEEEEGGCELRVKFSRSADAPAYKQGQNQLYNELNLGRREEYDVLDKRRGRDPEMGGKPRRKNPQEGLYNELQKDKMAEAYSEIGMKGERRRGKGHDGLYQGLSTATKDTYDALHMQALPPR

SEQ ID NO: 5 - protein, 612 aa, synthetic construct
MALPVTALLLPLALLLHAARPDIQMTQTTSSLSASLGDRVTISCRASQDISKYLNWYQQKPDGTVKLLIYHTSRLHSGVPSRFSGSGSGTDYSLTISNLEQEDIATYFCQQGNTLPYTFGGGTKLEITEETKKYQSEVQLQASGGGLVQGGGSLRVSCVASGLSFSYYGMGWFRQAPGKEREFVSAINWRGDTTSYADSVKGRFTISRENAKNTAYLQMNSLKPEDTAVYYCAARKYSAANVFKPNDYDYWGQGTQVTVSSSYTYNYEKEVKLQESGPGLVAPSQSLSVTCTVSGVSLPDYGVSWIRQPPRKGLEWLGVIWGSETTYYNSALKSRLTIIKDNSKSQVFLKMNSLQTDDTAIYYCAKHYYYGGSYAMDYWGQGTSVTVSSTTTPAPRPPTPAPTIASQPLSLRPEACRPAAGGAVHTRGLDFACDIYIWAPLAGTCGVLLLSLVITLYCKRGRKKLLYIFKQPFMRPVQTTQEEDGCSCRFPEEEEGGCELRVKFSRSADAPAYKQGQNQLYNELNLGRREEYDVLDKRRGRDPEMGGKPRRKNPQEGLYNELQKDKMAEAYSEIGMKGERRRGKGHDGLYQGLSTATKDTYDALHMQALPPR

SEQ ID NO: 6 - protein, 486 aa, synthetic construct
MALPVTALLLPLALLLHAARPDIQMTQTTSSLSASLGDRVTISCRASQDISKYLNWYQQKPDGTVKLLIYHTSRLHSGVPSRFSGSGSGTDYSLTISNLEQEDIATYFCQQGNTLPYTFGGGTKLEITGGGGSGGGGSGGGGSEVKLQESGPGLVAPSQSLSVTCTVSGVSLPDYGVSWIRQPPRKGLEWLGVIWGSETTYYNSALKSRLTIIKDNSKSQVFLKMNSLQTDDTAIYYCAKHYYYGGSYAMDYWGQGTSVTVSSTTTPAPRPPTPAPTIASQPLSLRPEACRPAAGGAVHTRGLDFACDIYIWAPLAGTCGVLLLSLVITLYCKRGRKKLLYIFKQPFMRPVQTTQEEDGCSCRFPEEEEGGCELRVKFSRSADAPAYKQGQNQLYNELNLGRREEYDVLDKRRGRDPEMGGKPRRKNPQEGLYNELQKDKMAEAYSEIGMKGERRRGKGHDGLYQGLSTATKDTYDALHMQALPPR

SEQ ID NO: 7 - protein, 369 aa, synthetic construct
MALPVTALLLPLALLLHAARPEVQLVESGGGLVQGGGSLRVSCVASGLSFSLYGMGWFRQAPGKEREFVAAINWRGDSTSYADSVKGRFTISRENAKNTAYLQMNSLKPEDTAVYYCAARKYSAANVFKPNDYDYWGQGTQVTVSSTTTPAPRPPTPAPTIASQPLSLRPEACRPAAGGAVHTRGLDFACDIYIWAPLAGTCGVLLLSLVITLYCKRGRKKLLYIFKQPFMRPVQTTQEEDGCSCRFPEEEEGGCELRVKFSRSADAPAYKQGQNQLYNELNLGRREEYDVLDKRRGRDPEMGGKPRRKNPQEGLYNELQKDKMAEAYSEIGMKGERRRGKGHDGLYQGLSTATKDTYDALHMQALPPR

SEQ ID NO: 8 - protein, 729 aa, synthetic construct
MALPVTALLLPLALLLHAARPDIQMTQTTSSLSASLGDRVTISCRASQDISKYLNWYQQKPDGTVKLLIYHTSRLHSGVPSRFSGSGSGTDYSLTISNLEQEDIATYFCQQGNTLPYTFGGGTKLEITGGGGSQVQLQQSGPGLVKPSQTLSLTCAISGDSVSSNSAAWNWIRQSPSRGLEWLGRTYYRSKWYNDYAVSVKSRITINPDTSKNQFSLQLNSVTPEDTAVYYCAREVTGDLEDAFDIWGQGTMVTVSSGSTSGSGKPGSGEGSTKGDIQMTQSPSSLSASVGDRVTITCRASQTIWSYLNWYQQRPGKAPNLLIYAASSLQSGVPSRFSGRGSGTDFTLTISSLQAEDFATYYCQQSYSIPQTFGQGTKLEIGGGGSEVKLQESGPGLVAPSQSLSVTCTVSGVSLPDYGVSWIRQPPRKGLEWLGVIWGSETTYYNSALKSRLTIIKDNSKSQVFLKMNSLQTDDTAIYYCAKHYYYGGSYAMDYWGQGTSVTVSSTTTPAPRPPTPAPTIASQPLSLRPEACRPAAGGAVHTRGLDFACDIYIWAPLAGTCGVLLLSLVITLYCKRGRKKLLYIFKQPFMRPVQTTQEEDGCSCRFPEEEEGGCELRVKFSRSADAPAYKQGQNQLYNELNLGRREEYDVLDKRRGRDPEMGGKPRRKNPQEGLYNELQKDKMAEAYSEIGMKGERRRGKGHDGLYQGLSTATKDTYDALHMQALPPR

SEQ ID NO: 9 - protein, 343 aa, synthetic construct
MALPVTALLLPLALLLHAARPDIVSDVPRDLEVVAATPTSLLISWSARLKVARYYRITYGETGGNSPVQEFTVPKNVYTATISGLKPGVDYTITVYAVTKMRDYRPISINYRTEIDKPSQTTTPAPRPPTPAPTIASQPLSLRPEACRPAAGGAVHTRGLDFACDIYIWAPLAGTCGVLLLSLVITLYCKRGRKKLLYIFKQPFMRPVQTTQEEDGCSCRFPEEEEGGCELRVKFSRSADAPAYKQGQNQLYNELNLGRREEYDVLDKRRGRDPEMGGKPRRKNPQEGLYNELQKDKMAEAYSEIGMKGERRRGKGHDGLYQGLSTATKDTYDALHMQALPPR

SEQ ID NO: 10 - protein, 595 aa, synthetic construct
MALPVTALLLPLALLLHAARPDIVSDVPRDLEVVAATPTSLLISWSARLKVARYYRITYGETGGNSPVQEFTVPKNVYTATISGLKPGVDYTITVYAVTKMRDYRPISINYRTEIDKPSQGGGGSDIQMTQSPSSLSASVGDRVTITCRASQDVNTAVAWYQQKPGKAPKLLIYSASFLYSGVPSRFSGSRSGTDFTLTISSLQPEDFATYYCQQHYTTPPTFGQGTKVEIKRTGGGGSGGGGSGGGGSEVQLVESGGGLVQPGGSLRLSCAASGFNIKDTYIHWVRQAPGKGLEWVARIYPTNGYTRYADSVKGRFTISADTSKNTAYLQMNSLRAEDTAVYYCSRWGGDGFYAMDYWGQGTLVTVSSAAATTTPAPRPPTPAPTIASQPLSLRPEACRPAAGGAVHTRGLDFACDIYIWAPLAGTCGVLLLSLVITLYCKRGRKKLLYIFKQPFMRPVQTTQEEDGCSCRFPEEEEGGCELRVKFSRSADAPAYKQGQNQLYNELNLGRREEYDVLDKRRGRDPEMGGKPRRKNPQEGLYNELQKDKMAEAYSEIGMKGERRRGKGHDGLYQGLSTATKDTYDALHMQALPPR

SEQ ID NO: 11 - protein, 595 aa, synthetic construct
MALPVTALLLPLALLLHAARPDIQMTQSPSSLSASVGDRVTITCRASQDVNTAVAWYQQKPGKAPKLLIYSASFLYSGVPSRFSGSRSGTDFTLTISSLQPEDFATYYCQQHYTTPPTFGQGTKVEIKRTGGGGSGGGGSGGGGSEVQLVESGGGLVQPGGSLRLSCAASGFNIKDTYIHWVRQAPGKGLEWVARIYPTNGYTRYADSVKGRFTISADTSKNTAYLQMNSLRAEDTAVYYCSRWGGDGFYAMDYWGQGTLVTVSSAAAGGGGSDIVSDVPRDLEVVAATPTSLLISWSARLKVARYYRITYGETGGNSPVQEFTVPKNVYTATISGLKPGVDYTITVYAVTKMRDYRPISINYRTEIDKPSQTTTPAPRPPTPAPTIASQPLSLRPEACRPAAGGAVHTRGLDFACDIYIWAPLAGTCGVLLLSLVITLYCKRGRKKLLYIFKQPFMRPVQTTQEEDGCSCRFPEEEEGGCELRVKFSRSADAPAYKQGQNQLYNELNLGRREEYDVLDKRRGRDPEMGGKPRRKNPQEGLYNELQKDKMAEAYSEIGMKGERRRGKGHDGLYQGLSTATKDTYDALHMQALPPR

SEQ ID NO: 12 - protein, 591 aa, synthetic construct
MALPVTALLLPLALLLHAARPDIQMTQSPSSLSASVGDRVTITCRASQDVNTAVAWYQQKPGKAPKLLIYSASFLYSGVPSRFSGSRSGTDFTLTISSLQPEDFATYYCQQHYTTPPTFGQGTKVEIKRTEETKKYQSDIVSDVPRDLEVVAATPTSLLISWSARLKVARYYRITYGETGGNSPVQEFTVPKNVYTATISGLKPGVDYTITVYAVTKMRDYRPISINYRTEIDKPSQSYTYNYEKEVQLVESGGGLVQPGGSLRLSCAASGFNIKDTYIHWVRQAPGKGLEWVARIYPTNGYTRYADSVKGRFTISADTSKNTAYLQMNSLRAEDTAVYYCSRWGGDGFYAMDYWGQGTLVTVSSAAATTTPAPRPPTPAPTIASQPLSLRPEACRPAAGGAVHTRGLDFACDIYIWAPLAGTCGVLLLSLVITLYCKRGRKKLLYIFKQPFMRPVQTTQEEDGCSCRFPEEEEGGCELRVKFSRSADAPAYKQGQNQLYNELNLGRREEYDVLDKRRGRDPEMGGKPRRKNPQEGLYNELQKDKMAEAYSEIGMKGERRRGKGHDGLYQGLSTATKDTYDALHMQALPPR

SEQ ID NO: 13 - protein, 491 aa, synthetic construct
MALPVTALLLPLALLLHAARPDIQMTQSPSSLSASVGDRVTITCRASQDVNTAVAWYQQKPGKAPKLLIYSASFLYSGVPSRFSGSRSGTDFTLTISSLQPEDFATYYCQQHYTTPPTFGQGTKVEIKRTGGGGSGGGGSGGGGSEVQLVESGGGLVQPGGSLRLSCAASGFNIKDTYIHWVRQAPGKGLEWVARIYPTNGYTRYADSVKGRFTISADTSKNTAYLQMNSLRAEDTAVYYCSRWGGDGFYAMDYWGQGTLVTVSSAAATTTPAPRPPTPAPTIASQPLSLRPEACRPAAGGAVHTRGLDFACDIYIWAPLAGTCGVLLLSLVITLYCKRGRKKLLYIFKQPFMRPVQTTQEEDGCSCRFPEEEEGGCELRVKFSRSADAPAYKQGQNQLYNELNLGRREEYDVLDKRRGRDPEMGGKPRRKNPQEGLYNELQKDKMAEAYSEIGMKGERRRGKGHDGLYQGLSTATKDTYDALHMQALPPR